European Patent Application EP 4 649 952 A1, published November 19, 2025. Title: KRAS Q16H specific T cell receptors and uses thereof. Applicant: HS Diagnomcis GmbH. Application EP. The sequence listing filed with the application follows.

SEQUENCE LISTING (23 sequences)

SEQ ID NO: 1 - protein, 15 aa, Homo sapiens
CALSEANQAGTALIF

SEQ ID NO: 2 - protein, 15 aa, Homo sapiens
CASSRKVPPVYGYTF

SEQ ID NO: 3 - protein, 15 aa, Homo sapiens
CALSEANQAGTALIF

SEQ ID NO: 4 - protein, 15 aa, Homo sapiens
CASSRRWPPTDTQYF

SEQ ID NO: 5 - protein, 15 aa, Homo sapiens
CALSEAKAAGNKLTF

SEQ ID NO: 6 - protein, 15 aa, Homo sapiens
CASSRKLPPTYGYTF

SEQ ID NO: 7 - protein, 15 aa, Homo sapiens
CALSEAGSSGSKLTF

SEQ ID NO: 8 - protein, 15 aa, Homo sapiens
CASSRRWPPTDTQYF

SEQ ID NO: 9 - protein, 15 aa, Homo sapiens
CALSEAGSSGSKLTF

SEQ ID NO: 10 - protein, 15 aa, Homo sapiens
CASSRKVPPVYGYTF

SEQ ID NO: 11 - protein, 114 aa, Homo sapiens
KVTQAQTEISVVEKEDVTLDCVYETRDTTYYLFWYKQPPSGELVFLIRRNSFDEQNEISGRYSWNFQKSTSSFNFTITASQVVDSAVYFCALSEANQAGTALIFGKGTTLSVSS

SEQ ID NO: 12 - protein, 114 aa, Homo sapiens
EAQVTQNPRYLITVTGKKLTVTCSQNMNHEYMSWYRQDPGLGLRQIYYSMNVEVTDKGDVPEGYKVSRKEKRNFPLILESPSPNQTSLYFCASSRKVPPVYGYTFGSGTRLTVV

SEQ ID NO: 13 - protein, 114 aa, Homo sapiens; identical to SEQ ID NO: 11

SEQ ID NO: 14 - protein, 114 aa, Homo sapiens
EAQVTQNPRYLITVTGKKLTVTCSQNMNHEYMSWYRQDPGLGLRQIYYSMNVEVTDKGDVPEGYKVSRKEKRNFPLILESPSPNQTSLYFCASSRRWPPTDTQYFGPGTRLTVL

SEQ ID NO: 15 - protein, 116 aa, Homo sapiens
AQKVTQAQTEISVVEKEDVTLDCVYETRDTTYYLFWYKQPPSGELVFLIRRNSFDEQNEISGRYSWNFQKSTSSFNFTITASQVVDSAVYFCALSEAKAAGNKLTFGGGTRVLVKP

SEQ ID NO: 16 - protein, 114 aa, Homo sapiens
EAQVTQNPRYLITVTGKKLTVTCSQNMNHEYMSWYRQDPGLGLRQIYYSMNVEVTDKGDVPEGYKVSRKEKRNFPLILESPSPNQTSLYFCASSRKLPPTYGYTFGSGTRLTVV

SEQ ID NO: 17 - protein, 116 aa, Homo sapiens
AQKVTQAQTEISVVEKEDVTLDCVYETRDTTYYLFWYKQPPSGELVFLIRRNSFDEQNEISGRYSWNFQKSTSSFNFTITASQVVDSAVYFCALSEAGSSGSKLTFGGGTRVLVKP

SEQ ID NO: 18 - protein, 114 aa, Homo sapiens; identical to SEQ ID NO: 14

SEQ ID NO: 19 - protein, 116 aa, Homo sapiens; identical to SEQ ID NO: 17

SEQ ID NO: 20 - protein, 114 aa, Homo sapiens; identical to SEQ ID NO: 12

SEQ ID NO: 21 - protein, 10 aa, synthetic construct
ILDTAGHEEY

SEQ ID NO: 22 - protein, 15 aa, synthetic construct
  VARIANT 7..9: note = XXX is NQA, GSS, or KAA
  VARIANT 11..12: note = XX is TA, SA, or NK
  VARIANT 14: note = X is I or T
CALSEAXXXGXXLXF

SEQ ID NO: 23 - protein, 15 aa, synthetic construct
  VARIANT 6..7: note = XX is KV, RW, RR or KL
  VARIANT 10..14: note = XXXXX is VYGYT, VYGDT, TDTQY, or TYGYT
CASSRXXPPXXXXXF